European Patent Application EP 4 458 986 A1, published November 6, 2024. Title: 多重PCR反应体系. Applicant: 迈克生物股份有限公司. The sequence listing filed with the application follows.

SEQUENCE LISTING (34 sequences)

SEQ ID NO: 1 - DNA, 40 bp, synthetic construct
  source 1..40: mol_type = other DNA
  misc_feature 28: note = modified with BHQ1
  misc_feature 40: note = modified with Spacer C3
  misc_feature 16: note = modified with CY5
ccctgggagctcatggaggtactggtcctgtcgacgcacg

SEQ ID NO: 2 - DNA, 55 bp, synthetic construct
  source 1..55: mol_type = other DNA
ttatttcatggaggtactggtcctgtcgaaatattgcagatccwacacctaacaa

SEQ ID NO: 3 - DNA, 42 bp, synthetic construct
  source 1..42: mol_type = other DNA
gctcccagggtttaacattaagcaagaagaggaaamgaagat

SEQ ID NO: 4 - DNA, 41 bp, synthetic construct
  source 1..41: mol_type = other DNA
  misc_feature 16: note = modified with VIC
  misc_feature 27: note = modified with BHQ2
  misc_feature 41: note = modified with Spacer C3
cgcaagtgaggcgactacgtgagcgatggacggaggcagga

SEQ ID NO: 5 - DNA, 37 bp, synthetic construct
  source 1..37: mol_type = other DNA
gcctcacttgcgaaaaagcaaccaacaacattcattg

SEQ ID NO: 6 - DNA, 42 bp, synthetic construct
  source 1..42: mol_type = other DNA
tttttctacgtgagcgatggaaagcaattcagcatcacagac

SEQ ID NO: 7 - DNA, 35 bp, synthetic construct
  source 1..35: mol_type = other DNA
gcctcacttgcgaaaataatcaggcacgagaacag

SEQ ID NO: 8 - DNA, 52 bp, synthetic construct
  source 1..52: mol_type = other DNA
tttttgactacgtgagcgatggacggaggaaaagactagcaacctccatggc

SEQ ID NO: 9 - DNA, 35 bp, synthetic construct
  source 1..35: mol_type = other DNA
  misc_feature 16: note = modified with FAM
  misc_feature 26: note = modified with BHQ1
  misc_feature 35: note = modified with Spacer C3
ccctgggagctcatggaggtactggtcctgtcgac

SEQ ID NO: 10 - DNA, 20 bp, synthetic construct
  source 1..20: mol_type = other DNA
  misc_feature 1: note = modified with BHQ1
  misc_feature 20: note = modified with FAM
agcgacggtgccgagagggt

SEQ ID NO: 11 - DNA, 55 bp, synthetic construct
  source 1..55: mol_type = other DNA
ttatttcatggaggtactggtcctgtcgaaatattgcagatactccacctcatca

SEQ ID NO: 12 - DNA, 42 bp, synthetic construct
  source 1..42: mol_type = other DNA
gctcccagggtttaacaggctgcaagaagaggactagaagat

SEQ ID NO: 13 - DNA, 47 bp, synthetic construct
  source 1..47: mol_type = other DNA
agcgacggtgccgagagggtaaatattgcagatactccacctcatca

SEQ ID NO: 14 - DNA, 29 bp, synthetic construct
  source 1..29: mol_type = other DNA
aacaggctgcaagaagaggactagaagat

SEQ ID NO: 15 - DNA, 33 bp, synthetic construct
  source 1..33: mol_type = other DNA
ttttttttttgatgaggtggagtatctgcaata

SEQ ID NO: 16 - DNA, 48 bp, synthetic construct
  source 1..48: mol_type = other DNA
ttatttggaggtactggtcctaaatattgcagatactccacctcatca

SEQ ID NO: 17 - DNA, 44 bp, synthetic construct
  source 1..44: mol_type = other DNA
gactgcagtcaatttaacaggctgcaagaagaggactagaagat

SEQ ID NO: 18 - DNA, 25 bp, synthetic construct
  source 1..25: mol_type = other DNA
gctcccagggaaagactgcagtcaa

SEQ ID NO: 19 - DNA, 40 bp, synthetic construct
  source 1..40: mol_type = other DNA
cgcattacaagttaaatattgcagatactccacctcatca

SEQ ID NO: 20 - DNA, 37 bp, synthetic construct
  source 1..37: mol_type = other DNA
ttatttggaggtactggtcctaaacgcattacaagtt

SEQ ID NO: 21 - DNA, 35 bp, synthetic construct; identical to SEQ ID NO: 9
  source 1..35: mol_type = other DNA
  misc_feature 16: note = modified with CY5
  misc_feature 28: note = modified with BHQ2
  misc_feature 35: note = modified with Spacer C3

SEQ ID NO: 22 - DNA, 44 bp, synthetic construct
  source 1..44: mol_type = other DNA
  misc_feature 1: note = modified with FAM
  misc_feature 15: note = modified with BHQ1
  misc_feature 44: note = modified with Spacer C3
ccacgtctcaactatgacactcctccgaccatccgcttcctcca

SEQ ID NO: 23 - DNA, 39 bp, synthetic construct
  source 1..39: mol_type = other DNA
ccacgtctcaactataaaagtctgaacgacctacactcc

SEQ ID NO: 24 - DNA, 34 bp, synthetic construct
  source 1..34: mol_type = other DNA
tggaggaagcggatgtttcccagcagctgacaca

SEQ ID NO: 25 - DNA, 48 bp, synthetic construct
  source 1..48: mol_type = other DNA
  misc_feature 20: note = modified with CY5
  misc_feature 33: note = modified with BHQ2
  misc_feature 48: note = modified with Spacer C3
ggccgtaatctgcactgcatcacatcgcccgctagcccgtccaatgcc

SEQ ID NO: 26 - DNA, 40 bp, synthetic construct
  source 1..40: mol_type = other DNA
ggccgtaatctgcactaaaagtctgaacgacctacactcc

SEQ ID NO: 27 - DNA, 34 bp, synthetic construct
  source 1..34: mol_type = other DNA
tagcgggcgatgtgatttcccagcagctgacaca

SEQ ID NO: 28 - DNA, 59 bp, synthetic construct
  source 1..59: mol_type = other DNA
  misc_feature 16: note = modified with FAM
  misc_feature 31: note = modified with BHQ2
  misc_feature 59: note = modified with Spacer C3
agacgcacggtgacatgtgtttgactcagttctgctgctgcccaccgtctggagtgcgt

SEQ ID NO: 29 - DNA, 34 bp, synthetic construct
  source 1..34: mol_type = other DNA
caccgtgcgtctaaatgatggacagcgtggacaa

SEQ ID NO: 30 - DNA, 44 bp, synthetic construct
  source 1..44: mol_type = other DNA
tttttcatgtgtttgactcagtttttcgaagagcatgagctgca

SEQ ID NO: 31 - DNA, 38 bp, synthetic construct
  source 1..38: mol_type = other DNA
caccgtgcgtctaaagtcaagatcacagattttgggcg

SEQ ID NO: 32 - DNA, 33 bp, synthetic construct
  source 1..33: mol_type = other DNA
ctgctgctgctttctggctgacctaaagccacc

SEQ ID NO: 33 - DNA, 36 bp, synthetic construct
  source 1..36: mol_type = other DNA
caccgtgcgtctaaaagattttgggctggccaaaca

SEQ ID NO: 34 - DNA, 36 bp, synthetic construct
  source 1..36: mol_type = other DNA
ctggagtgcgttttgcctccttctgcatggtattct